European Patent Specification EP 3 737 776 B1, published March 8, 2023. Title: ASSAY FOR DETECTING CHLAMYDIA TRACHOMATIS, NEISSERIA GONORRHOEAE, TRICHOMONAS VAGINALIS, AND MYCOPLASMA GENITALIUM. Applicant: ABBOTT LABORATORIES. The sequence listing filed with the application follows.

SEQUENCE LISTING (18 sequences)

SEQ ID NO: 1 - DNA, 21 bp, Artificial Sequence
  Synthetic
tcggagaccaatggcccgtaa

SEQ ID NO: 2 - DNA, 27 bp, Artificial Sequence
  Synthetic
gtttcgtgtctaaaccaaacgactctt

SEQ ID NO: 3 - DNA, 27 bp, Artificial Sequence
  Synthetic
agccagggagttaagctaaacggcgag

SEQ ID NO: 4 - DNA, 25 bp, Artificial Sequence
  Synthetic
ccggtttttgttcatccgccatatt

SEQ ID NO: 5 - DNA, 22 bp, Artificial Sequence
  Synthetic
cggctccttattcggtttgacc

SEQ ID NO: 6 - DNA, 18 bp, Artificial Sequence
  Synthetic
acaccgcccggaacccga

SEQ ID NO: 7 - DNA, 22 bp, Artificial Sequence
  Synthetic
ctttgccgaagtccttcggtta

SEQ ID NO: 8 - DNA, 20 bp, Artificial Sequence
  Synthetic
gagtagcgcaccctctcagg

SEQ ID NO: 9 - DNA, 23 bp, Artificial Sequence
  Synthetic
atgctctgggctgcacgcgtgct

SEQ ID NO: 10 - DNA, 24 bp, Artificial Sequence
  Synthetic
agcaatctggtagcttgcaaaagt

SEQ ID NO: 11 - DNA, 22 bp, Artificial Sequence
  Synthetic
ccctacaacccctatcctcaga

SEQ ID NO: 12 - DNA, 30 bp, Artificial Sequence
  Synthetic
cgaatgtgattccgtgtgtagtggcgagcg

SEQ ID NO: 13 - DNA, 28 bp, Artificial Sequence
  Synthetic
ctacagcagagttggcagcttcactttc

SEQ ID NO: 14 - DNA, 22 bp, Artificial Sequence
  Synthetic
gtctggcctttcagcaagtttc

SEQ ID NO: 15 - DNA, 25 bp, Artificial Sequence
  Synthetic
aagctgacgagttcatgagggcagg

SEQ ID NO: 16 - DNA, 22 bp, Artificial Sequence
  Synthetic
ggcaggttggtatcaaggttac

SEQ ID NO: 17 - DNA, 22 bp, Artificial Sequence
  Synthetic
cctaagggtgggaaaatagacc

SEQ ID NO: 18 - DNA, 28 bp, Artificial Sequence
  Synthetic
tttctgataggcactgactctctctgcc